European Patent Application EP 4 755 912 A1, published June 10, 2026. Title: 一种适用于免疫组化检测CD228的诊断抗体. Applicant: 山东博安生物技术股份有限公司. Application CN. The sequence listing filed with the application follows.

SEQUENCE LISTING (27 sequences)

SEQ ID NO: 1 - protein, 113 aa, synthetic construct
DPMLTQTASPVSAAVGSTVTINCQASQSVYNNNNLNWYQQKPGQPPKLLIYAASTLASGVPSRFKGSGSGTQFTLTISDVQCDDAATYYCLGAYDCSSADCGAFGGGTELEIL

SEQ ID NO: 2 - protein, 8 aa, synthetic construct
QSVYNNNN

SEQ ID NO: 3 - skipped

SEQ ID NO: 4 - protein, 13 aa, synthetic construct
LGAYDCSSADCGA

SEQ ID NO: 5 - protein, 109 aa, synthetic construct
QSLEESGGRLVKPDETLTLTCTVSGFSLSSYDMSWVRQAPGKGLQWIGAATAGGNTYHASWAKGRFTISKTSTTVDLKITSPTTEDTATYFCTRGLNIWGPGTLVTVSS

SEQ ID NO: 6 - protein, 8 aa, synthetic construct
GFSLSSYD

SEQ ID NO: 7 - protein, 7 aa, synthetic construct
ATAGGNT

SEQ ID NO: 8 - protein, 6 aa, synthetic construct
TRGLNI

SEQ ID NO: 9 - protein, 113 aa, synthetic construct
DPVLTQTASPVSAAVGGTITINCQASQSVYNNNQLSWFQQNPGQPPKRLIHSTSTLAPGVSSRFKGSGSGTQFTLTISDVQCDDAATYYCLGSYDCVSADCNAFGGGTEVVVK

SEQ ID NO: 10 - protein, 8 aa, synthetic construct
QSVYNNNQ

SEQ ID NO: 11 - skipped

SEQ ID NO: 12 - protein, 13 aa, synthetic construct
LGSYDCVSADCNA

SEQ ID NO: 13 - protein, 110 aa, synthetic construct
QEQLEESGGRLVTPGTPLTLTCTVSGFSLSTYAINWIRQAPGKGLEWIGIIGGNGATYYTNWAKGRFTISKTSTTVDLKITSPTIEDTATYFCARGTNFWGPGTLVTVSS

SEQ ID NO: 14 - protein, 8 aa, synthetic construct
GFTFSSYA

SEQ ID NO: 15 - protein, 7 aa, synthetic construct
IGGNGAT

SEQ ID NO: 16 - protein, 6 aa, synthetic construct
ARGTNF

SEQ ID NO: 17 - protein, 112 aa, synthetic construct
DVLMTQTPLTLSVTIGQPASISCKSSQSLLDSDGKTYLNWLLQRPGQSPKRLIYLVSKLDSGVPDRFTGSGSGTDFTLKISRVEAEDLGVYYCWQGTHFPRTFGGGTKLELK

SEQ ID NO: 18 - protein, 11 aa, synthetic construct
QSLLDSDGKTY

SEQ ID NO: 19 - skipped

SEQ ID NO: 20 - protein, 9 aa, synthetic construct
WQGTHFPRT

SEQ ID NO: 21 - protein, 115 aa, synthetic construct
EVQLQQSGAELVRPGTSVKVSCKASGYAFTNYLIEWIKQRPGQGLEWIGMINPGSGGTKYNEKFKGKATLTADKSSSTAYMQLSSLTSDDSAVYFCARDYYGYYWGQGTTLTVSS

SEQ ID NO: 22 - protein, 8 aa, synthetic construct
GYAFTNYL

SEQ ID NO: 23 - protein, 8 aa, synthetic construct
INPGSGGT

SEQ ID NO: 24 - protein, 8 aa, synthetic construct
ARDYYGYY

SEQ ID NO: 25 - protein, 323 aa, synthetic construct
GQPKAPSVFPLAPCCGDTPSSTVTLGCLVKGYLPEPVTVTWNSGTLTNGVRTFPSVRQSSGLYSLSSVVSVTSSSQPVTCNVAHPATNTKVDKTVAPSTCSKPTCPPPELLGGPSVFIFPPKPKDTLMISRTPEVTCVVVDVSQDDPEVQFTWYINNEQVRTARPPLREQQFNSTIRVVSTLPIAHQDWLRGKEFKCKVHNKALPAPIEKTISKARGQPLEPKVYTMGPPREELSSRSVSLTCMINGFYPSDISVEWEKNGKAEDNYKTTPAVLDSDGSYFLYSKLSVPTSEWQRGDVFTCSVMHEALHNHYTQKSISRSPGK

SEQ ID NO: 26 - protein, 104 aa, synthetic construct
GDPVAPTVLIFPPAADQVATGTVTIVCVANKYFPDVTVTWEVDGTTQTTGIENSKTPQNSADCTYNLSSTLTLTSTQYNSHKEYTCKVTQGTTSVVQSFNRGDC

SEQ ID NO: 27 - protein, 718 aa, synthetic construct
MRGPSGALWLLLALRTVLGGMEVRWCATSDPEQHKCGNMSEAFREAGIQPSLLCVRGTSADHCVQLIAAQEADAITLDGGAIYEAGKEHGLKPVVGEVYDQEVGTSYYAVAVVRRSSHVTIDTLKGVKSCHTGINRTVGWNVPVGYLVESGRLSVMGCDVLKAVSDYFGGSCVPGAGETSYSESLCRLCRGDSSGEGVCDKSPLERYYDYSGAFRCLAEGAGDVAFVKHSTVLENTDGKTLPSWGQALLSQDFELLCRDGSRADVTEWRQCHLARVPAHAVVVRADTDGGLIFRLLNEGQRLFSHEGSSFQMFSSEAYGQKDLLFKDSTSELVPIATQTYEAWLGHEYLHAMKGLLCDPNRLPPYLRWCVLSTPEIQKCGDMAVAFRRQRLKPEIQCVSAKSPQHCMERIQAEQVDAVTLSGEDIYTAGKTYGLVPAAGEHYAPEDSSNSYYVVAVVRRDSSHAFTLDELRGKRSCHAGFGSPAGWDVPVGALIQRGFIRPKDCDVLTAVSEFFNASCVPVNNPKNYPSSLCALCVGDEQGRNKCVGNSQERYYGYRGAFRCLVENAGDVAFVRHTTVFDNTNGHNSEPWAAELRSEDYELLCPNGARAEVSQFAACNLAQIPPHAVMVRPDTNIFTVYGLLDKAQDLFGDDHNKNGFKMFDSSNYHGQDLLFKDATVRAVPVGEKTTYRGWLGLDYVAALEGMSSQQHHHHHHHHHH